European Patent Application EP 4 393 515 A1, published July 3, 2024. Title: ANTI-CLDN-18.2 ANTIBODY-DRUG CONJUGATE AND USE THEREOF. Applicant: SHANGHAI JUNSHI BIOSCIENCES CO., LTD. The sequence listing filed with the application follows.

SEQUENCE LISTING (102 sequences)

SEQ ID NO: 1 - protein, 5 aa, synthetic construct
NFGMH

SEQ ID NO: 2 - protein, 17 aa, synthetic construct
CISSGSGTIYYADTVKG

SEQ ID NO: 3 - protein, 9 aa, synthetic construct
AYYGNGFSF

SEQ ID NO: 4 - protein, 10 aa, synthetic construct
SASSIFSYIF

SEQ ID NO: 5 - protein, 7 aa, synthetic construct
LTSKLAS

SEQ ID NO: 6 - protein, 8 aa, synthetic construct
HQWKITHT

SEQ ID NO: 7 - protein, 17 aa, synthetic construct
KSSQSLLNSGNQKNYLT

SEQ ID NO: 8 - protein, 7 aa, synthetic construct
WASTRES

SEQ ID NO: 9 - protein, 9 aa, synthetic construct
QNVYSYPLT

SEQ ID NO: 10 - protein, 5 aa, synthetic construct
NYGMN

SEQ ID NO: 11 - protein, 17 aa, synthetic construct
WINTYTGESTYADDFKG

SEQ ID NO: 12 - protein, 10 aa, synthetic construct
TLGYGNSLAY

SEQ ID NO: 13 - protein, 17 aa, synthetic construct
KSSQSLLNSGNQRNYLT

SEQ ID NO: 14 - protein, 7 aa, synthetic construct
WASTRES

SEQ ID NO: 15 - protein, 9 aa, synthetic construct
QNNYFYPFT

SEQ ID NO: 16 - protein, 5 aa, synthetic construct
SFGVS

SEQ ID NO: 17 - protein, 16 aa, synthetic construct
AIWAGGNRNYNSALMS

SEQ ID NO: 18 - protein, 9 aa, synthetic construct
GSYGSSFAN

SEQ ID NO: 19 - protein, 17 aa, synthetic construct
KSSQSLLNSGNQKNYLT

SEQ ID NO: 20 - protein, 7 aa, synthetic construct
WASTRDS

SEQ ID NO: 21 - protein, 9 aa, synthetic construct
QNAYFYPFT

SEQ ID NO: 22 - protein, 5 aa, synthetic construct
NYGMN

SEQ ID NO: 23 - protein, 17 aa, synthetic construct
WINTYTGESTYADDFKG

SEQ ID NO: 24 - protein, 9 aa, synthetic construct
SYNGNSLPY

SEQ ID NO: 25 - protein, 17 aa, synthetic construct
KSSQSLLNSGNQKNYLT

SEQ ID NO: 26 - protein, 7 aa, synthetic construct
WASTRES

SEQ ID NO: 27 - protein, 9 aa, synthetic construct
QNDYSYPLT

SEQ ID NO: 28 - protein, 5 aa, synthetic construct
SYGMS

SEQ ID NO: 29 - protein, 17 aa, synthetic construct
TISGGDSYTYYPDSVRG

SEQ ID NO: 30 - protein, 9 aa, synthetic construct
SYNGNSLPY

SEQ ID NO: 31 - protein, 17 aa, synthetic construct
KSSQSLLNSGNQKNYLT

SEQ ID NO: 32 - protein, 7 aa, synthetic construct
WASTRES

SEQ ID NO: 33 - protein, 9 aa, synthetic construct
QNTYSFPLT

SEQ ID NO: 34 - protein, 5 aa, synthetic construct
NYGMN

SEQ ID NO: 35 - protein, 17 aa, synthetic construct
WINTYTGEPTYADDFKG

SEQ ID NO: 36 - skipped

SEQ ID NO: 37 - protein, 5 aa, synthetic construct
NYLIE

SEQ ID NO: 38 - protein, 17 aa, synthetic construct
VINPGSGGTNYNEKFKG

SEQ ID NO: 39 - protein, 11 aa, synthetic construct
PHDGYYFWFAY

SEQ ID NO: 40 - protein, 17 aa, synthetic construct
WINTYTGESTYADGFTG

SEQ ID NO: 41 - protein, 17 aa, synthetic construct
SISSGSGTIYYADSVKG

SEQ ID NO: 42 - protein, 118 aa, synthetic construct
DVQLVESGGGLVQPGGSRKLSCAASGFTLNNFGMHWVRQAPEKGLEWVACISSGSGTIYYADTVKGRFTISRDNPKNTLFLQMTSLRSEDTAMYYCARAYYGNGFSFWGQGTLVTVSS

SEQ ID NO: 43 - protein, 105 aa, synthetic construct
QIVLTQSPTLMSASPGEKVTMTCSASSIFSYIFWSQQKPRSSPKPWIYLTSKLASGVPVRFSGSGSGTSYSLTISTMEAEDAATYYCHQWKITHTFGAGTKLELK

SEQ ID NO: 44 - protein, 113 aa, synthetic construct
DIVMTQSPSSLTVTAGEKVTMSCKSSQSLLNSGNQKNYLTWYQQKPGQPPKLLIYWASTRESGVPDRFTGSGSGTDFTLTISSVQAEDLAIYYCQNVYSYPLTFGAGTKLEIK

SEQ ID NO: 45 - protein, 118 aa, synthetic construct
QIQLVQSGPELKKPGETVKISCKASGYTFTNYGMNWVKQAPGKGLKWMGWINTYTGESTYADDFKGRFAFSSETSARTAYLQINNLKNEDMATYFCATLGYGNSLAYWGQGTLVTVSS

SEQ ID NO: 46 - protein, 113 aa, synthetic construct
DIVMTQYPSFLTVTTGEKVTMSCKSSQSLLNSGNQRNYLTWYQQKPGQPPKLLIYWASTRESGVPDRFAGSGSGTDFTLTISSVQAEDLAIYYCQNNYFYPFTFGSGTKLEVK

SEQ ID NO: 47 - protein, 117 aa, synthetic construct
QVQLKESGPGLVAPSQSLSITCTVSGFSLTSFGVSWVRQPPGKGLEWLGAIWAGGNRNYNSALMSRLSISKDNSKSQVFLKMTSLQTDDTAIYYCARGSYGSSFANWGQGTLVTVSS

SEQ ID NO: 48 - protein, 113 aa, synthetic construct
DIVMTQSPSFLTVTAGEKVTMSCKSSQSLLNSGNQKNYLTWYQQKPGQPPKLLIYWASTRDSGVPDRFTGSGSGTDFTLTITSVQAEDLAVFYCQNAYFYPFTFGSGTKLEIK

SEQ ID NO: 49 - protein, 118 aa, synthetic construct
QIQLVQSGPELKKPGETVKISCKASGYTFTNYGMNWVKQAPGKGLKWMGWINTYTGESTYADDFKGRFAFSSETSARTAYLQINNLKNEGMATYFCARSYNGNSLPYWGQGTLVTVSS

SEQ ID NO: 50 - protein, 113 aa, synthetic construct
DIVMTQSPSFLTVTAGEKVTMSCKSSQSLLNSGNQKNYLTWYQQKPGQPPKLLIYWASTRESGVPDRFTGSGSGTDFTLTISSVQAEDLAVYYCQNDYSYPLTFGAGTKLELK

SEQ ID NO: 51 - protein, 118 aa, synthetic construct
EVKLVESGGGLVKPGGSLKLSCAASGFTFSSYGMSWVRQTPEKRLECVATISGGDSYTYYPDSVRGRFTISRDIAKNNLYLQMSSLRSEDTALYYCARSYNGNSLPYWGQGTLVTVSS

SEQ ID NO: 52 - protein, 113 aa, synthetic construct
DIVMTQSPSSLTVTAGEKVTMSCKSSQSLLNSGNQKNYLTWYQQKPGQPPKLLIYWASTRESGVPDRFTGSGSGIDFTLTISSVQAEDLAFYYCQNTYSFPLTFGAGTRLDLK

SEQ ID NO: 53 - protein, 111 aa, synthetic construct
QIQLVQSGPELKKPGETVKISCKASGYTFTNYGMNWVKQAPGKGLKWMGWINTYTGEPTYADDFKGRFAFSLETSASTAYLQINNLKNEDTATYFCARGYWGQGTTLTVSS

SEQ ID NO: 54 - protein, 120 aa, synthetic construct
QVQLQQSGAELVRPGTSVKVSCKASGYAFTNYLIEWVKQRPGQGLEWIGVINPGSGGTNYNEKFKGKATLTADKSSSTAYMQLSSLTSDDSAVYFCARPHDGYYFWFAYWGQGTLVTVSS

SEQ ID NO: 55 - protein, 118 aa, synthetic construct
QIQLVQSGSELKKPGESVKVSCKASGYTFTNYGMNWVRQAPGQGLEWMGWINTYTGESTYADGFTGRFVFSSDTSARTAYLQISSLKAEDTAVYFCATLGYGNSLAYWGQGTLVTVSS

SEQ ID NO: 56 - protein, 113 aa, synthetic construct
DIVMTQSPDSLAVSLGERATINCKSSQSLLNSGNQRNYLTWYQQKPGQPPKLLIYWASTRESGVPDRFSGSGSGTDFTLTISSLQAEDVAVYYCQNNYFYPFTFGQGTKLEIK

SEQ ID NO: 57 - protein, 118 aa, synthetic construct
QVQLVQSGSELKKPGESVKVSCKASGYTFTNYGMNWVRQAPGQGLEWMGWINTYTGESTYADGFTGRFVFSMDTSASTAYLQISSLKAEDMAMYFCATLGYGNSLAYWGQGTLVTVSS

SEQ ID NO: 58 - protein, 118 aa, synthetic construct
EVQLVESGGGLVKPGGSLRLSCAASGFTFSSYGMSWVRQAPGKGLEWVSTISGGDSYTYYPDSVRGRFTISRDNAKNSLYLQMNSLRAEDTAVYYCARSYNGNSLPYWGQGTLVTVSS

SEQ ID NO: 59 - protein, 118 aa, synthetic construct
EVQLVESGGGLVKPGGSLRLSCAASGFTFSSYGMSWVRQAPGKGLESVSTISGGDSYTYYPDSVRGRFTISRDIAKNSLYLQMNSLRAEDTAVYYCARSYNGNSLPYWGQGTLVTVSS

SEQ ID NO: 60 - protein, 118 aa, synthetic construct
EVQLVESGGGLVQPGGSLRLSCAASGFTLNNFGMHWVRQAPGKGLEWVSSISSGSGTIYYADSVKGRFTISRDNPKNSLYLQMNSLRAEDTAVYYCARAYYGNGFSFWGQGTLVTVSS

SEQ ID NO: 61 - protein, 113 aa, synthetic construct
DIVMTQSPDSLAVSLGERATINCKSSQSLLNSGNQKNYLTWYQQKPGQPPKLLIYWASTRESGVPDRFSGSGSGTDFTLTISSLQAEDVAVYYCQNVYSYPLTFGQGTKLEIK

SEQ ID NO: 62 - protein, 17 aa, synthetic construct
  MUTAGEN 1: note = X is C or S
  MUTAGEN 14: note = X is T or S
XISSGSGTIYYADXVKG

SEQ ID NO: 63 - protein, 17 aa, synthetic construct
  MUTAGEN 14: note = X is D or G
  MUTAGEN 16: note = X is K or T
WINTYTGESTYADXFXG

SEQ ID NO: 64 - protein, 448 aa, synthetic construct
EVQLVESGGGLVQPGGSLRLSCAASGFTLNNFGMHWVRQAPGKGLEWVSSISSGSGTIYYADSVKGRFTISRDNPKNSLYLQMNSLRAEDTAVYYCARAYYGNGFSFWGQGTLVTVSSASTKGPSVFPLAPSSKSTSGGTAALGCLVKDYFPEPVTVSWNSGALTSGVHTFPAVLQSSGLYSLSSVVTVPSSSLGTQTYICNVNHKPSNTKVDKKVEPKSCDKTHTCPPCPAPELLGGPSVFLFPPKPKDTLMISRTPEVTCVVVDVSHEDPEVKFNWYVDGVEVHNAKTKPREEQYNSTYRVVSVLTVLHQDWLNGKEYKCKVSNKALPAPIEKTISKAKGQPREPQVYTLPPSRDELTKNQVSLTCLVKGFYPSDIAVEWESNGQPENNYKTTPPVLDSDGSFFLYSKLTVDKSRWQQGNVFSCSVMHEALHNHYTQKSLSLSPGK

SEQ ID NO: 65 - protein, 220 aa, synthetic construct
DIVMTQSPDSLAVSLGERATINCKSSQSLLNSGNQKNYLTWYQQKPGQPPKLLIYWASTRESGVPDRFSGSGSGTDFTLTISSLQAEDVAVYYCQNVYSYPLTFGQGTKLEIKRTVAAPSVFIFPPSDEQLKSGTASVVCLLNNFYPREAKVQWKVDNALQSGNSQESVTEQDSKDSTYSLSSTLTLSKADYEKHKVYACEVTHQGLSSPVTKSFNRGEC

SEQ ID NO: 66 - DNA, 1347 bp, synthetic construct
  source 1..1347: mol_type = other DNA
gaggtgcagctggtggagagcggcggcggcctggtgcagcccggcggcagcctgagactgagctgcgccgccagcggcttcaccctgaacaacttcggcatgcactgggtgagacaggcccccggcaagggcctggagtgggtgagctccatcagcagcggcagcggcaccatctactacgccgacagcgtgaagggcagattcaccatcagcagagacaaccccaagaacagcctgtacctgcagatgaacagcctgagagccgaggacaccgccgtgtactactgcgccagagcctactacggcaacggcttcagcttctggggccagggcaccctggtgaccgtgagcagcgctagcaccaagggcccatccgtcttccccctggcaccctcctccaagagcacctctgggggcacagcggccctgggctgcctggtcaaggactacttccccgaaccggtgacggtgtcgtggaactcaggcgccctgaccagcggcgtgcacaccttcccggctgtcctacagtcctcaggactctactccctcagcagcgtggtgaccgtgccctccagcagcttgggcacccagacctacatctgcaacgtgaatcacaagcccagcaacaccaaggtggacaagaaagttgagcccaaatcttgtgacaaaactcacacatgcccaccgtgcccagcacctgaactcctggggggaccgtcagtcttcctcttccccccaaaacccaaggacaccctcatgatctcccggacccctgaggtcacatgcgtggtggtggacgtgagccacgaagaccctgaggtcaagttcaactggtacgtggacggcgtggaggtgcataatgccaagacaaagccgcgggaggagcagtacaacagcacgtaccgtgtggtcagcgtcctcaccgtcctgcaccaggactggctgaatggcaaggagtacaagtgcaaggtctccaacaaagccctcccagcccccatcgagaaaaccatctccaaagccaaagggcagccccgagaaccacaggtgtacaccctgcccccatcccgggacgagctgaccaagaaccaggtcagcctgacctgcctggtcaaaggcttctatcccagcgacatcgccgtggagtgggagagcaatgggcagccggagaacaactacaagaccacgcctcccgtgctggactccgacggctccttcttcctctatagcaagctcaccgtggacaagagcaggtggcagcaggggaacgtcttctcatgctccgtgatgcatgaggctctgcacaaccactacacgcagaagtccctctccctgtctccgggtaaatga

SEQ ID NO: 67 - DNA, 663 bp, synthetic construct
  source 1..663: mol_type = other DNA
gacatcgtgatgacccagagccccgacagcctggccgtgagcctgggcgagagagccaccatcaactgcaagagcagccagagcctgctgaacagcggcaaccagaagaactacctgacctggtaccagcagaagcccggccagccccccaagctgctgatctactgggccagcaccagagagagcggcgtgcccgacagattcagcggcagcggcagcggcaccgacttcaccctgaccatcagcagcctgcaggccgaggacgtggccgtgtactactgccagaacgtgtacagctaccccctgaccttcggccagggcaccaagctggagatcaagcgaactgtggctgcaccatctgtcttcatcttcccgccatctgatgagcagttgaaatctggaactgcctctgttgtgtgcctgctgaataacttctatcccagagaggccaaagtacagtggaaggtggataacgccctccaatcgggtaactcccaggagagtgtcacagagcaggacagcaaggacagcacctacagcctcagcagcaccctgacgctgagcaaagcagactacgagaaacacaaagtctacgcctgcgaagtcacccatcagggcctgagctcgcccgtcacaaagagcttcaacaggggagagtgttag

SEQ ID NO: 68 - protein, 448 aa, synthetic construct
QIQLVQSGSELKKPGESVKVSCKASGYTFTNYGMNWVRQAPGQGLEWMGWINTYTGESTYADGFTGRFVFSSDTSARTAYLQISSLKAEDTAVYFCATLGYGNSLAYWGQGTLVTVSSASTKGPSVFPLAPSSKSTSGGTAALGCLVKDYFPEPVTVSWNSGALTSGVHTFPAVLQSSGLYSLSSVVTVPSSSLGTQTYICNVNHKPSNTKVDKKVEPKSCDKTHTCPPCPAPELLGGPSVFLFPPKPKDTLMISRTPEVTCVVVDVSHEDPEVKFNWYVDGVEVHNAKTKPREEQYNSTYRVVSVLTVLHQDWLNGKEYKCKVSNKALPAPIEKTISKAKGQPREPQVYTLPPSRDELTKNQVSLTCLVKGFYPSDIAVEWESNGQPENNYKTTPPVLDSDGSFFLYSKLTVDKSRWQQGNVFSCSVMHEALHNHYTQKSLSLSPGK

SEQ ID NO: 69 - protein, 220 aa, synthetic construct
DIVMTQSPDSLAVSLGERATINCKSSQSLLNSGNQRNYLTWYQQKPGQPPKLLIYWASTRESGVPDRFSGSGSGTDFTLTISSLQAEDVAVYYCQNNYFYPFTFGQGTKLEIKRTVAAPSVFIFPPSDEQLKSGTASVVCLLNNFYPREAKVQWKVDNALQSGNSQESVTEQDSKDSTYSLSSTLTLSKADYEKHKVYACEVTHQGLSSPVTKSFNRGEC

SEQ ID NO: 70 - DNA, 1347 bp, synthetic construct
  source 1..1347: mol_type = other DNA
cagatccagctggtgcagagcggcagcgagctgaagaagcccggcgagagcgtgaaggtgagctgcaaggccagcggctacaccttcaccaactacggcatgaactgggtgagacaggcccccggccagggcctggagtggatgggctggatcaacacctacaccggcgagagcacctacgccgacggcttcaccggcagattcgtgttcagcagcgacaccagcgccagaaccgcctacctgcagatcagcagcctgaaggccgaggacaccgccgtgtacttctgcgccaccctgggctacggcaacagcctggcctactggggccagggcaccctggtgaccgtgagcagcgctagcaccaagggcccatccgtcttccccctggcaccctcctccaagagcacctctgggggcacagcggccctgggctgcctggtcaaggactacttccccgaaccggtgacggtgtcgtggaactcaggcgccctgaccagcggcgtgcacaccttcccggctgtcctacagtcctcaggactctactccctcagcagcgtggtgaccgtgccctccagcagcttgggcacccagacctacatctgcaacgtgaatcacaagcccagcaacaccaaggtggacaagaaagttgagcccaaatcttgtgacaaaactcacacatgcccaccgtgcccagcacctgaactcctggggggaccgtcagtcttcctcttccccccaaaacccaaggacaccctcatgatctcccggacccctgaggtcacatgcgtggtggtggacgtgagccacgaagaccctgaggtcaagttcaactggtacgtggacggcgtggaggtgcataatgccaagacaaagccgcgggaggagcagtacaacagcacgtaccgtgtggtcagcgtcctcaccgtcctgcaccaggactggctgaatggcaaggagtacaagtgcaaggtctccaacaaagccctcccagcccccatcgagaaaaccatctccaaagccaaagggcagccccgagaaccacaggtgtacaccctgcccccatcccgggacgagctgaccaagaaccaggtcagcctgacctgcctggtcaaaggcttctatcccagcgacatcgccgtggagtgggagagcaatgggcagccggagaacaactacaagaccacgcctcccgtgctggactccgacggctccttcttcctctatagcaagctcaccgtggacaagagcaggtggcagcaggggaacgtcttctcatgctccgtgatgcatgaggctctgcacaaccactacacgcagaagtccctctccctgtctccgggtaaatga

SEQ ID NO: 71 - DNA, 663 bp, synthetic construct
  source 1..663: mol_type = other DNA
gacatcgtgatgacccagagccccgacagcctggccgtgagcctgggcgagagagccaccatcaactgcaagagcagccagagcctgctgaacagcggcaaccagagaaactacctgacctggtaccagcagaagcccggccagccccccaagctgctgatctactgggccagcaccagagagagcggcgtgcccgacagattcagcggcagcggcagcggcaccgacttcaccctgaccatcagcagcctgcaggccgaggacgtggccgtgtactactgccagaacaactacttctaccccttcaccttcggccagggcaccaagctggagatcaagcgaactgtggctgcaccatctgtcttcatcttcccgccatctgatgagcagttgaaatctggaactgcctctgttgtgtgcctgctgaataacttctatcccagagaggccaaagtacagtggaaggtggataacgccctccaatcgggtaactcccaggagagtgtcacagagcaggacagcaaggacagcacctacagcctcagcagcaccctgacgctgagcaaagcagactacgagaaacacaaagtctacgcctgcgaagtcacccatcagggcctgagctcgcccgtcacaaagagcttcaacaggggagagtgttag

SEQ ID NO: 72 - protein, 17 aa, synthetic construct
YISSGSGTIYYADSVKG

SEQ ID NO: 73 - protein, 9 aa, synthetic construct
AYYGNAFSF

SEQ ID NO: 74 - protein, 17 aa, synthetic construct
TISGGDSYTYYPDSVKG

SEQ ID NO: 75 - protein, 9 aa, synthetic construct
SYNANSLPY

SEQ ID NO: 76 - protein, 118 aa, synthetic construct
EVQLVESGGGLVQPGGSLRLSCAASGFTLNNFGMHWVRQAPGKGLEWVSYISSGSGTIYYADSVKGRFTISRDNPKNSLYLQMNSLRAEDTAVYYCARAYYGNAFSFWGQGTLVTVSS

SEQ ID NO: 77 - protein, 113 aa, synthetic construct
DIVMTQSPSSLAVSLGERATINCKSSQSLLNSGNQKNYLTWYQQKPGQPPKLLIYWASTRESGVPDRFSGSGSGTDFTLTISSLQAEDVAVYYCQNVYSYPLTFGQGTKLEIK

SEQ ID NO: 78 - protein, 118 aa, synthetic construct
EVQLVESGGGLVQPGGSLRLSCAASGFTLNNFGMHWVRQAPGKGLEWVSYISSGSGTIYYADSVKGRFTISRDNPKNSLYLQMNSLRAEDTAVYYCARAYYGNGFSFWGQGTLVTVSS

SEQ ID NO: 79 - protein, 118 aa, synthetic construct
QIQLVQSGSELKKPGASVKVSCKASGYTFTNYGMNWVRQAPGQGLEWMGWINTYTGESTYADGFTGRFVFSSDTSARTAYLQISSLKAEDTAVYFCATLGYGNSLAYWGQGTLVTVSS

SEQ ID NO: 80 - protein, 113 aa, synthetic construct
DIVMTQSPDSLAVTTGERATINCKSSQSLLNSGNQRNYLTWYQQKPGQPPKLLIYWASTRESGVPDRFSGSGSGTDFTLTISSLQAEDVAVYYCQNNYFYPFTFGQGTKLEIK

SEQ ID NO: 81 - protein, 113 aa, synthetic construct
DIVMTQSPDFLAVSLGERATINCKSSQSLLNSGNQKNYLTWYQQKPGQPPKLLIYWASTRDSGVPDRFSGSGSGTDFTLTISSLQAEDVAVYYCQNAYFYPFTFGPGTKVDIK

SEQ ID NO: 82 - protein, 118 aa, synthetic construct
EVQLVESGGGLVKPGGSLRLSCAASGFTFSSYGMSWVRQAPGKGLEWVSTISGGDSYTYYPDSVKGRFTISRDIAKNSLYLQMNSLRAEDTAVYYCARSYNANSLPYWGQGTLVTVSS

SEQ ID NO: 83 - protein, 118 aa, synthetic construct
EVQLVESGGGLVKPGGSLRLSCAASGFTFSSYGMSWVRQAPGKGLEWVSTISGGDSYTYYPDSVKGRFTISRDNAKNSLYLQMNSLRAEDTAVYYCARSYNGNSLPYWGQGTLVTVSS

SEQ ID NO: 84 - protein, 448 aa, synthetic construct
EVQLVESGGGLVQPGGSLRLSCAASGFTLNNFGMHWVRQAPGKGLEWVSYISSGSGTIYYADSVKGRFTISRDNPKNSLYLQMNSLRAEDTAVYYCARAYYGNAFSFWGQGTLVTVSSASTKGPSVFPLAPSSKSTSGGTAALGCLVKDYFPEPVTVSWNSGALTSGVHTFPAVLQSSGLYSLSSVVTVPSSSLGTQTYICNVNHKPSNTKVDKKVEPKSCDKTHTCPPCPAPELLGGPSVFLFPPKPKDTLMISRTPEVTCVVVDVSHEDPEVKFNWYVDGVEVHNAKTKPREEQYNSTYRVVSVLTVLHQDWLNGKEYKCKVSNKALPAPIEKTISKAKGQPREPQVYTLPPSRDELTKNQVSLTCLVKGFYPSDIAVEWESNGQPENNYKTTPPVLDSDGSFFLYSKLTVDKSRWQQGNVFSCSVMHEALHNHYTQKSLSLSPGK

SEQ ID NO: 85 - protein, 220 aa, synthetic construct; identical to SEQ ID NO: 65

SEQ ID NO: 86 - protein, 448 aa, synthetic construct; identical to SEQ ID NO: 84

SEQ ID NO: 87 - protein, 220 aa, synthetic construct
DIVMTQSPSSLAVSLGERATINCKSSQSLLNSGNQKNYLTWYQQKPGQPPKLLIYWASTRESGVPDRFSGSGSGTDFTLTISSLQAEDVAVYYCQNVYSYPLTFGQGTKLEIKRTVAAPSVFIFPPSDEQLKSGTASVVCLLNNFYPREAKVQWKVDNALQSGNSQESVTEQDSKDSTYSLSSTLTLSKADYEKHKVYACEVTHQGLSSPVTKSFNRGEC

SEQ ID NO: 88 - protein, 448 aa, synthetic construct
EVQLVESGGGLVQPGGSLRLSCAASGFTLNNFGMHWVRQAPGKGLEWVSYISSGSGTIYYADSVKGRFTISRDNPKNSLYLQMNSLRAEDTAVYYCARAYYGNGFSFWGQGTLVTVSSASTKGPSVFPLAPSSKSTSGGTAALGCLVKDYFPEPVTVSWNSGALTSGVHTFPAVLQSSGLYSLSSVVTVPSSSLGTQTYICNVNHKPSNTKVDKKVEPKSCDKTHTCPPCPAPELLGGPSVFLFPPKPKDTLMISRTPEVTCVVVDVSHEDPEVKFNWYVDGVEVHNAKTKPREEQYNSTYRVVSVLTVLHQDWLNGKEYKCKVSNKALPAPIEKTISKAKGQPREPQVYTLPPSRDELTKNQVSLTCLVKGFYPSDIAVEWESNGQPENNYKTTPPVLDSDGSFFLYSKLTVDKSRWQQGNVFSCSVMHEALHNHYTQKSLSLSPGK

SEQ ID NO: 89 - protein, 220 aa, synthetic construct; identical to SEQ ID NO: 65

SEQ ID NO: 90 - protein, 448 aa, synthetic construct
QIQLVQSGSELKKPGASVKVSCKASGYTFTNYGMNWVRQAPGQGLEWMGWINTYTGESTYADGFTGRFVFSSDTSARTAYLQISSLKAEDTAVYFCATLGYGNSLAYWGQGTLVTVSSASTKGPSVFPLAPSSKSTSGGTAALGCLVKDYFPEPVTVSWNSGALTSGVHTFPAVLQSSGLYSLSSVVTVPSSSLGTQTYICNVNHKPSNTKVDKKVEPKSCDKTHTCPPCPAPELLGGPSVFLFPPKPKDTLMISRTPEVTCVVVDVSHEDPEVKFNWYVDGVEVHNAKTKPREEQYNSTYRVVSVLTVLHQDWLNGKEYKCKVSNKALPAPIEKTISKAKGQPREPQVYTLPPSRDELTKNQVSLTCLVKGFYPSDIAVEWESNGQPENNYKTTPPVLDSDGSFFLYSKLTVDKSRWQQGNVFSCSVMHEALHNHYTQKSLSLSPGK

SEQ ID NO: 91 - protein, 220 aa, synthetic construct
DIVMTQSPDSLAVTTGERATINCKSSQSLLNSGNQRNYLTWYQQKPGQPPKLLIYWASTRESGVPDRFSGSGSGTDFTLTISSLQAEDVAVYYCQNNYFYPFTFGQGTKLEIKRTVAAPSVFIFPPSDEQLKSGTASVVCLLNNFYPREAKVQWKVDNALQSGNSQESVTEQDSKDSTYSLSSTLTLSKADYEKHKVYACEVTHQGLSSPVTKSFNRGEC

SEQ ID NO: 92 - protein, 448 aa, synthetic construct
QVQLVQSGSELKKPGESVKVSCKASGYTFTNYGMNWVRQAPGQGLEWMGWINTYTGESTYADGFTGRFVFSMDTSASTAYLQISSLKAEDMAMYFCATLGYGNSLAYWGQGTLVTVSSASTKGPSVFPLAPSSKSTSGGTAALGCLVKDYFPEPVTVSWNSGALTSGVHTFPAVLQSSGLYSLSSVVTVPSSSLGTQTYICNVNHKPSNTKVDKKVEPKSCDKTHTCPPCPAPELLGGPSVFLFPPKPKDTLMISRTPEVTCVVVDVSHEDPEVKFNWYVDGVEVHNAKTKPREEQYNSTYRVVSVLTVLHQDWLNGKEYKCKVSNKALPAPIEKTISKAKGQPREPQVYTLPPSRDELTKNQVSLTCLVKGFYPSDIAVEWESNGQPENNYKTTPPVLDSDGSFFLYSKLTVDKSRWQQGNVFSCSVMHEALHNHYTQKSLSLSPGK

SEQ ID NO: 93 - protein, 220 aa, synthetic construct; identical to SEQ ID NO: 69

SEQ ID NO: 94 - protein, 448 aa, synthetic construct; identical to SEQ ID NO: 68

SEQ ID NO: 95 - protein, 220 aa, synthetic construct
DIVMTQSPDFLAVSLGERATINCKSSQSLLNSGNQKNYLTWYQQKPGQPPKLLIYWASTRDSGVPDRFSGSGSGTDFTLTISSLQAEDVAVYYCQNAYFYPFTFGPGTKVDIKRTVAAPSVFIFPPSDEQLKSGTASVVCLLNNFYPREAKVQWKVDNALQSGNSQESVTEQDSKDSTYSLSSTLTLSKADYEKHKVYACEVTHQGLSSPVTKSFNRGEC

SEQ ID NO: 96 - protein, 448 aa, synthetic construct; identical to SEQ ID NO: 92

SEQ ID NO: 97 - protein, 220 aa, synthetic construct; identical to SEQ ID NO: 69

SEQ ID NO: 98 - protein, 448 aa, synthetic construct
EVQLVESGGGLVKPGGSLRLSCAASGFTFSSYGMSWVRQAPGKGLEWVSTISGGDSYTYYPDSVKGRFTISRDIAKNSLYLQMNSLRAEDTAVYYCARSYNANSLPYWGQGTLVTVSSASTKGPSVFPLAPSSKSTSGGTAALGCLVKDYFPEPVTVSWNSGALTSGVHTFPAVLQSSGLYSLSSVVTVPSSSLGTQTYICNVNHKPSNTKVDKKVEPKSCDKTHTCPPCPAPELLGGPSVFLFPPKPKDTLMISRTPEVTCVVVDVSHEDPEVKFNWYVDGVEVHNAKTKPREEQYNSTYRVVSVLTVLHQDWLNGKEYKCKVSNKALPAPIEKTISKAKGQPREPQVYTLPPSRDELTKNQVSLTCLVKGFYPSDIAVEWESNGQPENNYKTTPPVLDSDGSFFLYSKLTVDKSRWQQGNVFSCSVMHEALHNHYTQKSLSLSPGK

SEQ ID NO: 99 - protein, 220 aa, synthetic construct; identical to SEQ ID NO: 69

SEQ ID NO: 100 - protein, 448 aa, synthetic construct
EVQLVESGGGLVKPGGSLRLSCAASGFTFSSYGMSWVRQAPGKGLEWVSTISGGDSYTYYPDSVKGRFTISRDNAKNSLYLQMNSLRAEDTAVYYCARSYNGNSLPYWGQGTLVTVSSASTKGPSVFPLAPSSKSTSGGTAALGCLVKDYFPEPVTVSWNSGALTSGVHTFPAVLQSSGLYSLSSVVTVPSSSLGTQTYICNVNHKPSNTKVDKKVEPKSCDKTHTCPPCPAPELLGGPSVFLFPPKPKDTLMISRTPEVTCVVVDVSHEDPEVKFNWYVDGVEVHNAKTKPREEQYNSTYRVVSVLTVLHQDWLNGKEYKCKVSNKALPAPIEKTISKAKGQPREPQVYTLPPSRDELTKNQVSLTCLVKGFYPSDIAVEWESNGQPENNYKTTPPVLDSDGSFFLYSKLTVDKSRWQQGNVFSCSVMHEALHNHYTQKSLSLSPGK

SEQ ID NO: 101 - protein, 220 aa, synthetic construct; identical to SEQ ID NO: 69

SEQ ID NO: 102 - protein, 448 aa, synthetic construct
EVQLVESGGGLVKPGGSLRLSCAASGFTFSSYGMSWVRQAPGKGLEWVSTISGGDSYTYYPDSVRGRFTISRDNAKNSLYLQMNSLRAEDTAVYYCARSYNGNSLPYWGQGTLVTVSSASTKGPSVFPLAPSSKSTSGGTAALGCLVKDYFPEPVTVSWNSGALTSGVHTFPAVLQSSGLYSLSSVVTVPSSSLGTQTYICNVNHKPSNTKVDKKVEPKSCDKTHTCPPCPAPELLGGPSVFLFPPKPKDTLMISRTPEVTCVVVDVSHEDPEVKFNWYVDGVEVHNAKTKPREEQYNSTYRVVSVLTVLHQDWLNGKEYKCKVSNKALPAPIEKTISKAKGQPREPQVYTLPPSRDELTKNQVSLTCLVKGFYPSDIAVEWESNGQPENNYKTTPPVLDSDGSFFLYSKLTVDKSRWQQGNVFSCSVMHEALHNHYTQKSLSLSPGK